European Patent Specification EP 3 452 089 B1, published December 24, 2025. Title: BISPECIFIC BINDING PROTEINS AND USES THEREOF. Applicant: MedImmune, LLC. The sequence listing filed with the application follows.

SEQUENCE LISTING (97 sequences)

SEQ ID NO: 1 - protein, 711 aa, Artificial Sequence
  Description of Artificial Sequence: Synthetic       polypeptide
DIQMTQSPSSLSASVGDRVTITCRASQSINSYLDWYQQKPGKAPKLLIYAASSLQSGVPSRFSGSGSGTDFTLTISSLQPEDFATYYCQQYYSTPFTFGCGTKVEIKGGGGSGGGGSGGGGSGGGGSQVQLVESGGGVVQPGRSLRLSCAASGFTFSSYGMHWVRQAPGKCLEWVAVIWYDGSNKYYADSVKGRFTISRDNSKNTLYLQMNSLRAEDTAVYYCARDPRGATLYYYYYGMDVWGQGTTVTVSSGGGGSGGGGSEVQLVESGGGLVQPGGSLRLSCAASGFTFSDYGMHWVRQAPGKGLEWVAYISSGSYTIYSADSVKGRFTISRDNAKNSLYLQMNSLRAEDTAVYYCARRAPNSFYEYYFDYWGQGTTVTVSSASTKGPSVFPLAPCSRSTSESTAALGCLVKDYFPEPVTVSWNSGALTSGVHTFPAVLQSSGLYSLSSVVTVPSSSLGTKTYTCNVDHKPSNTKVDKRVESKYGPPCPPCPAPEFLGGPSVFLFPPKPKDTLMISRTPEVTCVVVDVSQEDPEVQFNWYVDGVEVHNAKTKPREEQFNSTYRVVSVLTVLHQDWLNGKEYKCKVSNKGLPSSIEKTISKAKGQPREPQVYTLPPSQEEMTKNQVSLTCLVKGFYPSDIAVEWESNGQPENNYKTTPPVLDSDGSFFLYSRLTVDKSRWQEGNVFSCSVMHEALHNHYTQKSLSLSLGK

SEQ ID NO: 2 - protein, 219 aa, Artificial Sequence
  Description of Artificial Sequence: Synthetic       polypeptide
QIVLTQSPATLSLSPGERATLSCSASSKHTNLYWSRHMYWYQQKPGQAPRLLIYLTSNRATGIPARFSGSGSGTDFTLTISSLEPEDFAVYYCQQWSSNPFTFGQGTKLEIKRTVAAPSVFIFPPSDEQLKSGTASVVCLLNNFYPREAKVQWKVDNALQSGNSQESVTEQDSKDSTYSLSSTLTLSKADYEKHKVYACEVTHQGLSSPVTKSFNRGEC

SEQ ID NO: 3 - protein, 711 aa, Artificial Sequence
  Description of Artificial Sequence: Synthetic       polypeptide
EVQLVESGGGLVQPGGSLRLSCAASGFTFSDYGMHWVRQAPGKGLEWVAYISSGSYTIYSADSVKGRFTISRDNAKNSLYLQMNSLRAEDTAVYYCARRAPNSFYEYYFDYWGQGTTVTVSSASTKGPSVFPLAPCSRSTSESTAALGCLVKDYFPEPVTVSWNSGALTSGVHTFPAVLQSSGLYSLSSVVTVPSSSLGTKTYTCNVDHKPSNTKVDKRVESKYGPPCPPCPAPEFLGGPSVFLFPPKPKDTLMISRTPEVTCVVVDVSQEDPEVQFNWYVDGVEVHNAKTKPREEQFNSTYRVVSVLTVLHQDWLNGKEYKCKVSNKGLPSSIEKTISKAKGQPREPQVYTLPPSQEEMTKNQVSLTCLVKGFYPSDIAVEWESNGQPENNYKTTPPVLDSDGSFFLYSRLTVDKSRWQEGNVFSCSVMHEALHNHYTQKSLSLSLGKGGGGSGGGGSDIQMTQSPSSLSASVGDRVTITCRASQSINSYLDWYQQKPGKAPKLLIYAASSLQSGVPSRFSGSGSGTDFTLTISSLQPEDFATYYCQQYYSTPFTFGCGTKVEIKGGGGSGGGGSGGGGSGGGGSQVQLVESGGGVVQPGRSLRLSCAASGFTFSSYGMHWVRQAPGKCLEWVAVIWYDGSNKYYADSVKGRFTISRDNSKNTLYLQMNSLRAEDTAVYYCARDPRGATLYYYYYGMDVWGQGTTVTVSS

SEQ ID NO: 4 - protein, 219 aa, Artificial Sequence; identical to SEQ ID NO: 2
  Description of Artificial Sequence: Synthetic       polypeptide

SEQ ID NO: 5 - protein, 721 aa, Artificial Sequence
  Description of Artificial Sequence: Synthetic       polypeptide
EVQLVESGGGLVQPGGSLRLSCAASGFTFSDYGMHWVRQAPGKGLEWVAYISSGSYTIYSADSVKGRFTISRDNAKNSLYLQMNSLRAEDTAVYYCARRAPNSFYEYYFDYWGQGTTVTVSSASTKGPSVFPLAPCSRSTSESTAALGCLVKDYFPEPVTVSWNSGALTSGVHTFPAVLQSSGLYSLSSVVTVPSSSLGTKTYTCNVDHKPSNTKVDKRVESKYGPPCPPCPAPEFLGGPSVFLFPPKPKDTLMISRTPEVTCVVVDVSQEDPEVQFNWYVDGVEVHNAKTKPREEQFNSTYRVVSVLTVLHQDWLNGKEYKCKVSNKGLPSSIEKTISKAKGQPREPQVYTLPPSQEEMTKNQVSLTCLVKGFYPSDIAVEWESNGGGGSGGGGSDIQMTQSPSSLSASVGDRVTITCRASQSINSYLDWYQQKPGKAPKLLIYAASSLQSGVPSRFSGSGSGTDFTLTISSLQPEDFATYYCQQYYSTPFTFGCGTKVEIKGGGGSGGGGSGGGGSGGGGSQVQLVESGGGVVQPGRSLRLSCAASGFTFSSYGMHWVRQAPGKCLEWVAVIWYDGSNKYYADSVKGRFTISRDNSKNTLYLQMNSLRAEDTAVYYCARDPRGATLYYYYYGMDVWGQGTTVTVSSGGGGSGGGGSGQPENNYKTTPPVLDSDGSFFLYSRLTVDKSRWQEGNVFSCSVMHEALHNHYTQKSLSLSLGK

SEQ ID NO: 6 - protein, 219 aa, Artificial Sequence; identical to SEQ ID NO: 2
  Description of Artificial Sequence: Synthetic       polypeptide

SEQ ID NO: 7 - protein, 219 aa, Artificial Sequence; identical to SEQ ID NO: 2
  Description of Artificial Sequence: Synthetic       polypeptide

SEQ ID NO: 8 - DNA, 610 bp, Artificial Sequence
  Description of Artificial Sequence: Synthetic polynucleotide
cgagagagccaccctgagctgctccgcctcctccaagcacaccaacctgtactggtcccggcacatgtactggtatcagcagaagcccggccaggcccctcggctgctgatctacctgacctctaaccgggccaccggcatccctgccagattctccggctctggctccggcaccgacttcaccctgaccatctccagcctggaacccgaggacttcgccgtgtactactgccagcagtggtcctccaaccccttcaccttcggccagggcaccaagctggaaatcaagcgtacggtggctgcaccatctgtcttcatcttcccgccatctgatgagcagttgaaatctggaactgcctctgttgtgtgcctgctgaataacttctatcccagagaggccaaagtacagtggaaggtggataacgccctccaatcgggtaactcccaggagagtgtcacagagcaggacagcaaggacagcacctacagcctcagcagcaccctgacgctgagcaaagcagactacgagaaacacaaagtctacgcctgcgaagtcacccatcagggcctgagctcgcccgtcacaaagagcttcaacaggggagagtgt

SEQ ID NO: 9 - protein, 452 aa, Artificial Sequence
  Description of Artificial Sequence: Synthetic       polypeptide
EVQLVESGGGLVQPGGSLRLSCAASGFTFSDYGMHWVRQAPGKGLEWVAYISSGSYTIYSADSVKGRFTISRDNAKNSLYLQMNSLRAEDTAVYYCARRAPNSFYEYYFDYWGQGTTVTVSSASTKGPSVFPLAPSSKSTSGGTAALGCLVKDYFPEPVTVSWNSGALTSGVHTFPAVLQSSGLYSLSSVVTVPSSSLGTQTYICNVNHKPSNTKVDKRVEPKSCDKTHTCPPCPAPEFEGGPSVFLFPPKPKDTLMISRTPEVTCVVVDVSHEDPEVKFNWYVDGVEVHNAKTKPREEQYNSTYRVVSVLTVLHQDWLNGKEYKCKVSNKALPASIEKTISKAKGQPREPQVCTLPPSREEMTKNQVSLSCAVKGFYPSDIAVEWESNGQPENNYKTTPPVLDSDGSFFLVSKLTVDKSRWQQGNVFSCSVMHEALHNHYTQKSLSLSPGK

SEQ ID NO: 10 - DNA, 1356 bp, Artificial Sequence
  Description of Artificial Sequence: Synthetic polynucleotide
gaggtgcagctggtggaatccggcggaggactggtgcagcctggcggctccctgagactgtcttgcgccgcctccggcttcacattctccgactacggcatgcactgggtccgacaggcccctggaaagggcctggaatgggtggcctacatctcctccggctcctacaccatctactccgccgactccgtgaagggccggttcaccatctcccgggacaacgccaagaactccctgtacctgcagatgaactccctgcgggccgaggacacagccgtgtactactgtgccagacgggcccctaactccttctacgagtactacttcgactactggggccagggcaccaccgtgaccgtgtcctctgctagcaccaaaggtccgagcgtttttccgctggcaccgagcagcaaaagcacctctggtggcaccgcagcactgggttgtctggtgaaagattattttccggaaccggttaccgtttcttggaatagcggtgcactgaccagcggtgttcatacctttccggcagttctgcagagcagcggtctgtatagcctgtctagcgttgttaccgttccgagcagcagcctgggcacccagacctatatttgcaatgtgaatcataaaccgagcaatacaaaagttgataaacgcgttgaaccgaaaagctgtgacaaaactcacacgtgcccaccgtgcccagcacctgagttcgaggggggaccgtcagtcttcctcttccccccaaaacccaaggacaccctcatgatctcccggacccctgaggtcacatgcgtggtggtggacgtgagccacgaagaccctgaggtcaagttcaactggtacgtggacggcgtggaggtgcataatgccaagacaaagccgcgggaggagcagtacaacagcacgtaccgtgtggtcagcgtcctcaccgtcctgcaccaggactggctgaatggcaaggagtacaagtgcaaggtctccaacaaagccctcccagccagcatcgagaaaaccatctccaaagccaaagggcagccccgagaaccacaggtctgcaccctgcccccatcccgggaggagatgaccaagaaccaggtcagcctgagctgcgcggtcaaaggcttctatcccagcgacatcgccgtggagtgggagagcaatgggcagccggagaacaactacaagaccacgcctcccgtgctggactccgacggctccttcttcctcgttagcaagctcaccgtggacaagagcaggtggcagcaggggaacgtcttctcatgctccgtgatgcatgaggctctgcacaaccactacacgcagaagagcctctccctgtctccgggtaaa

SEQ ID NO: 11 - DNA, 639 bp, Artificial Sequence
  Description of Artificial Sequence: Synthetic polynucleotide
gacatccagatgacccagtctccatcctccctgtctgcatctgtaggagacagagtcaccatcacttgccgggcaagtcagagcattaacagctatttagattggtatcagcagaaaccagggaaagcccctaaactcctgatctatgctgcatccagtttgcaaagtggggtcccatcaaggttcagtggcagtggatctgggacagatttcactctcaccatcagcagtctgcaacctgaagattttgcaacttactactgtcaacagtattacagtactccattcactttcggccctgggaccaaagtggaaatcaaaggtcagcccaaggcggccccctcggtcactctgttcccgccctgctctgaggagcttcaagccaacaaggccacactggtgtgtctcataagtgacttctacccgggagccgtgacagtggcctggaaggcagatagcagccccgtcaaggcgggagtggagaccaccacaccctccaaacaaagcaacaacaagtacgcggccagcagctacctgagcctgacgcctgagcagtggaagtcccacagaagctacagctgccaggtcacgcatgaagggagcaccgtggagaagacagtggcccctacagaagtgtca

SEQ ID NO: 12 - protein, 455 aa, Artificial Sequence
  Description of Artificial Sequence: Synthetic       polypeptide
QVQLVESGGGVVQPGRSLRLSCAASGFTFSSYGMHWVRQAPGKGLEWVAVIWYDGSNKYYADSVKGRFTISRDNSKNTLYLQMNSLRAEDTAVYYCARDPRGATLYYYYYGMDVWGQGTTVTVSSASTKGPSVCPLAPSSKSTSGGTAALGCLVKDYFPEPVTVSWNSGALTSGVHTFPAVLQSSGLYSLSSVVTVPSSSLGTQTYICNVNHKPSNTKVDKRVEPKSVDKTHTCPPCPAPEFEGGPSVFLFPPKPKDTLMISRTPEVTCVVVDVSHEDPEVKFNWYVDGVEVHNAKTKPREEQYNSTYRVVSVLTVLHQDWLNGKEYKCKVSNKALPASIEKTISKAKGQPREPQVYTLPPCREEMTKNQVSLWCLVKGFYPSDIAVEWESNGQPENNYKTTPPVLDSDGSFFLYSKLTVDKSRWQQGNVFSCSVMHEALHNHYTQKSLSLSPGK

SEQ ID NO: 13 - DNA, 1365 bp, Artificial Sequence
  Description of Artificial Sequence: Synthetic polynucleotide
caggtgcagctggtggagtctgggggaggcgtggtccagcctgggaggtccctgagactctcctgtgcagcgtctggattcaccttcagtagctatggcatgcactgggtccgccaggctccaggcaaggggctggagtgggtggcagttatatggtatgatggaagtaataaatactatgcagactccgtgaagggccgattcaccatctccagagacaattccaagaacacgctgtatctgcaaatgaacagcctgagagccgaggacacggctgtgtattactgtgcgagagatccgaggggagctaccctttactactactactacggtatggacgtctggggccaagggaccacggtcaccgtctcctcagcgtcgaccaaaggtccgagcgtgtgcccgctggcaccgagcagcaaaagcacctctggtggcaccgcagcactgggttgtctggtgaaagattattttccggaaccggttaccgtttcttggaatagcggtgcactgaccagcggtgttcatacctttccggcagtcctgcagagcagcggtctgtatagcctgtctagcgttgttaccgttccgagcagcagcctgggcacccagacctatatttgcaatgtgaatcataaaccgagcaataccaaagttgataaacgcgttgaaccgaaaagcgtggacaaaactcacacgtgcccaccgtgcccagcacctgagttcgaggggggaccgtcagtcttcctcttccccccaaaacccaaggacaccctcatgatctcccggacccctgaggtcacatgcgtggtggtggacgtgagccacgaagaccctgaggtcaagttcaactggtacgtggacggcgtggaggtgcataatgccaagacaaagccgcgggaggagcagtacaacagcacgtaccgtgtggtcagcgtcctcaccgtcctgcaccaggactggctgaatggcaaggagtacaagtgcaaggtctccaacaaagccctcccagccagcatcgagaaaaccatctccaaagccaaagggcagccccgagaaccacaggtctacaccctgcccccatgccgggaggagatgaccaagaaccaggtcagcctgtggtgcctggtcaaaggcttctatcccagcgacatcgccgtggagtgggagagcaatgggcagccggagaacaactacaagaccacgcctcccgtgctggactccgacggctccttcttcctctatagcaagctcaccgtggacaagagcaggtggcagcaggggaacgtcttctcatgctccgtgatgcatgaggctctgcacaaccactacacgcagaagagcttaagcctgtctccgggtaaa

SEQ ID NO: 14 - protein, 710 aa, Artificial Sequence
  Description of Artificial Sequence: Synthetic       polypeptide
DIQMTQSPSSLSASVGDRVTITCRASQSINSYLDWYQQKPGKAPKLLIYAASSLQSGVPSRFSGSGSGTDFTLTISSLQPEDFATYYCQQYYSTPFTFGCGTKVEIKGGGGSGGGGSGGGGSGGGGSQVQLVESGGGVVQPGRSLRLSCAASGFTFSSYGMHWVRQAPGKCLEWVAVIWYDGSNKYYADSVKGRFTISRDNSKNTLYLQMNSLRAEDTAVYYCARDPRGATLYYYYYGMDVWGQGTTVTVSSGGGGSGGGGSEVQLVESGGGLVQPGGSLRLSCAASGFTFSRYWMSWVRQAPGKGLEWVANIKQDGSEKYYVDSVKGRFTISRDNAKNSLYLQMNSLRAEDTAVYYCAREGGWFGELAFDYWGQGTLVTVSSASTKGPSVFPLAPCSRSTSESTAALGCLVKDYFPEPVTVSWNSGALTSGVHTFPAVLQSSGLYSLSSVVTVPSSSLGTKTYTCNVDHKPSNTKVDKRVESKYGPPCPPCPAPEFLGGPSVFLFPPKPKDTLMISRTPEVTCVVVDVSQEDPEVQFNWYVDGVEVHNAKTKPREEQFNSTYRVVSVLTVLHQDWLNGKEYKCKVSNKGLPSSIEKTISKAKGQPREPQVYTLPPSQEEMTKNQVSLTCLVKGFYPSDIAVEWESNGQPENNYKTTPPVLDSDGSFFLYSRLTVDKSRWQEGNVFSCSVMHEALHNHYTQKSLSLSLGK

SEQ ID NO: 15 - protein, 215 aa, Artificial Sequence
  Description of Artificial Sequence: Synthetic       polypeptide
EIVLTQSPGTLSLSPGERATLSCRASQRVSSSYLAWYQQKPGQAPRLLIYDASSRATGIPDRFSGSGSGTDFTLTISRLEPEDFAVYYCQQYGSLPWTFGQGTKVEIKRTVAAPSVFIFPPSDEQLKSGTASVVCLLNNFYPREAKVQWKVDNALQSGNSQESVTEQDSKDSTYSLSSTLTLSKADYEKHKVYACEVTHQGLSSPVTKSFNRGEC

SEQ ID NO: 16 - protein, 710 aa, Artificial Sequence
  Description of Artificial Sequence: Synthetic       polypeptide
EVQLVESGGGLVQPGGSLRLSCAASGFTFSRYWMSWVRQAPGKGLEWVANIKQDGSEKYYVDSVKGRFTISRDNAKNSLYLQMNSLRAEDTAVYYCAREGGWFGELAFDYWGQGTLVTVSSASTKGPSVFPLAPCSRSTSESTAALGCLVKDYFPEPVTVSWNSGALTSGVHTFPAVLQSSGLYSLSSVVTVPSSSLGTKTYTCNVDHKPSNTKVDKRVESKYGPPCPPCPAPEFLGGPSVFLFPPKPKDTLMISRTPEVTCVVVDVSQEDPEVQFNWYVDGVEVHNAKTKPREEQFNSTYRVVSVLTVLHQDWLNGKEYKCKVSNKGLPSSIEKTISKAKGQPREPQVYTLPPSQEEMTKNQVSLTCLVKGFYPSDIAVEWESNGQPENNYKTTPPVLDSDGSFFLYSRLTVDKSRWQEGNVFSCSVMHEALHNHYTQKSLSLSLGKGGGGSGGGGSDIQMTQSPSSLSASVGDRVTITCRASQSINSYLDWYQQKPGKAPKLLIYAASSLQSGVPSRFSGSGSGTDFTLTISSLQPEDFATYYCQQYYSTPFTFGCGTKVEIKGGGGSGGGGSGGGGSGGGGSQVQLVESGGGVVQPGRSLRLSCAASGFTFSSYGMHWVRQAPGKCLEWVAVIWYDGSNKYYADSVKGRFTISRDNSKNTLYLQMNSLRAEDTAVYYCARDPRGATLYYYYYGMDVWGQGTTVTVSS

SEQ ID NO: 17 - protein, 215 aa, Artificial Sequence; identical to SEQ ID NO: 15
  Description of Artificial Sequence: Synthetic       polypeptide

SEQ ID NO: 18 - protein, 720 aa, Artificial Sequence
  Description of Artificial Sequence: Synthetic       polypeptide
EVQLVESGGGLVQPGGSLRLSCAASGFTFSRYWMSWVRQAPGKGLEWVANIKQDGSEKYYVDSVKGRFTISRDNAKNSLYLQMNSLRAEDTAVYYCAREGGWFGELAFDYWGQGTLVTVSSASTKGPSVFPLAPCSRSTSESTAALGCLVKDYFPEPVTVSWNSGALTSGVHTFPAVLQSSGLYSLSSVVTVPSSSLGTKTYTCNVDHKPSNTKVDKRVESKYGPPCPPCPAPEFLGGPSVFLFPPKPKDTLMISRTPEVTCVVVDVSQEDPEVQFNWYVDGVEVHNAKTKPREEQFNSTYRVVSVLTVLHQDWLNGKEYKCKVSNKGLPSSIEKTISKAKGQPREPQVYTLPPSQEEMTKNQVSLTCLVKGFYPSDIAVEWESNGGGGSGGGGSDIQMTQSPSSLSASVGDRVTITCRASQSINSYLDWYQQKPGKAPKLLIYAASSLQSGVPSRFSGSGSGTDFTLTISSLQPEDFATYYCQQYYSTPFTFGCGTKVEIKGGGGSGGGGSGGGGSGGGGSQVQLVESGGGVVQPGRSLRLSCAASGFTFSSYGMHWVRQAPGKCLEWVAVIWYDGSNKYYADSVKGRFTISRDNSKNTLYLQMNSLRAEDTAVYYCARDPRGATLYYYYYGMDVWGQGTTVTVSSGGGGSGGGGSGQPENNYKTTPPVLDSDGSFFLYSRLTVDKSRWQEGNVFSCSVMHEALHNHYTQKSLSLSLGK

SEQ ID NO: 19 - protein, 215 aa, Artificial Sequence; identical to SEQ ID NO: 15
  Description of Artificial Sequence: Synthetic       polypeptide

SEQ ID NO: 20 - protein, 250 aa, Artificial Sequence
  Description of Artificial Sequence: Synthetic       polypeptide
EVQLLESGGGLVQPGGSLRLSCAASGFTFSSYAMSWVRQAPGKCLEWVSAISGSGGSTYYADSVKGRFTISRDNSKNTLYLQMNSLRAEDTAVYYCARGSYGTYYGNYFEYWGRGTLVTVSSGGGGSGGGGSGGGGSGGGGSQTVLTQPPSVSVAPGKTASISCGGDNIGGKSVHWYQQKPGQAPVLVIYYDSDRPSGIPQRFSGSNSGNTATLTIHRVEAGDEADYYCQVLDRRSDHWLFGCGTKLTVL

SEQ ID NO: 21 - protein, 709 aa, Artificial Sequence
  Description of Artificial Sequence: Synthetic       polypeptide
EVQLVESGGGLVQPGGSLRLSCAASGFTFSDYGMHWVRQAPGKGLEWVAYISSGSYTIYSADSVKGRFTISRDNAKNSLYLQMNSLRAEDTAVYYCARRAPNSFYEYYFDYWGQGTTVTVSSASTKGPSVFPLAPCSRSTSESTAALGCLVKDYFPEPVTVSWNSGALTSGVHTFPAVLQSSGLYSLSSVVTVPSSSLGTKTYTCNVDHKPSNTKVDKRVESKYGPPCPPCPAPEFLGGPSVFLFPPKPKDTLMISRTPEVTCVVVDVSQEDPEVQFNWYVDGVEVHNAKTKPREEQFNSTYRVVSVLTVLHQDWLNGKEYKCKVSNKGLPSSIEKTISKAKGQPREPQVYTLPPSQEEMTKNQVSLTCLVKGFYPSDIAVEWESNGQPENNYKTTPPVLDSDGSFFLYSRLTVDKSRWQEGNVFSCSVMHEALHNHYTQKSLSLSLGKGGGGSGGGGSEVQLLESGGGLVQPGGSLRLSCAASGFTFSSYAMSWVRQAPGKCLEWVSAISGSGGSTYYADSVKGRFTISRDNSKNTLYLQMNSLRAEDTAVYYCARGSYGTYYGNYFEYWGRGTLVTVSSGGGGSGGGGSGGGGSGGGGSQTVLTQPPSVSVAPGKTASISCGGDNIGGKSVHWYQQKPGQAPVLVIYYDSDRPSGIPQRFSGSNSGNTATLTIHRVEAGDEADYYCQVLDRRSDHWLFGCGTKLTVL

SEQ ID NO: 22 - protein, 719 aa, Artificial Sequence
  Description of Artificial Sequence: Synthetic       polypeptide
EVQLVESGGGLVQPGGSLRLSCAASGFTFSDYGMHWVRQAPGKGLEWVAYISSGSYTIYSADSVKGRFTISRDNAKNSLYLQMNSLRAEDTAVYYCARRAPNSFYEYYFDYWGQGTTVTVSSASTKGPSVFPLAPCSRSTSESTAALGCLVKDYFPEPVTVSWNSGALTSGVHTFPAVLQSSGLYSLSSVVTVPSSSLGTKTYTCNVDHKPSNTKVDKRVESKYGPPCPPCPAPEFLGGPSVFLFPPKPKDTLMISRTPEVTCVVVDVSQEDPEVQFNWYVDGVEVHNAKTKPREEQFNSTYRVVSVLTVLHQDWLNGKEYKCKVSNKGLPSSIEKTISKAKGQPREPQVYTLPPSQEEMTKNQVSLTCLVKGFYPSDIAVEWESNGGGGSGGGGSEVQLLESGGGLVQPGGSLRLSCAASGFTFSSYAMSWVRQAPGKCLEWVSAISGSGGSTYYADSVKGRFTISRDNSKNTLYLQMNSLRAEDTAVYYCARGSYGTYYGNYFEYWGRGTLVTVSSGGGGSGGGGSGGGGSGGGGSQTVLTQPPSVSVAPGKTASISCGGDNIGGKSVHWYQQKPGQAPVLVIYYDSDRPSGIPQRFSGSNSGNTATLTIHRVEAGDEADYYCQVLDRRSDHWLFGCGTKLTVLGGGGSGGGGSGQPENNYKTTPPVLDSDGSFFLYSRLTVDKSRWQEGNVFSCSVMHEALHNHYTQKSLSLSLGK

SEQ ID NO: 23 - protein, 219 aa, Artificial Sequence; identical to SEQ ID NO: 2
  Description of Artificial Sequence: Synthetic       polypeptide

SEQ ID NO: 24 - protein, 709 aa, Artificial Sequence; identical to SEQ ID NO: 21
  Description of Artificial Sequence: Synthetic       polypeptide

SEQ ID NO: 25 - protein, 452 aa, Artificial Sequence
  Description of Artificial Sequence: Synthetic       polypeptide
EVQLVESGGGLVQPGGSLRLSCAASGFTFSDYGMHWVRQAPGKGLEWVAYISSGSYTIYSADSVKGRFTISRDNAKNSLYLQMNSLRAEDTAVYYCARRAPNSFYEYYFDYWGQGTTVTVSSASTKGPSVFPLAPSSKSTSGGTAALGCLVKDYFPEPVTVSWNSGALTSGVHTFPAVLQSSGLYSLSSVVTVPSSSLGTQTYICNVNHKPSNTKVDKRVEPKSCDKTHTCPPCPAPELLGGPSVFLFPPKPKDTLMISRTPEVTCVVVDVSHEDPEVKFNWYVDGVEVHNAKTKPREEQYNSTYRVVSVLTVLHQDWLNGKEYKCKVSNKALPAPIEKTISKAKGQPREPQVCTLPPSREEMTKNQVSLSCAVKGFYPSDIAVEWESNGQPENNYKTTPPVLDSDGSFFLVSKLTVDKSRWQQGNVFSCSVMHEALHNHYTQKSLSLSPGK

SEQ ID NO: 26 - protein, 214 aa, Artificial Sequence
  Description of Artificial Sequence: Synthetic       polypeptide
QTVLTQPPSVSVAPGKTASISCGGDNIGGKSVHWYQQKPGQAPVLVIYYDSDRPSGIPQRFSGSNSGNTATLTIHRVEAGDEADYYCQVLDRRSDHWLFGGGTKLTVLGQPKAAPSVTLFPPCSEELQANKATLVCLISDFYPGAVTVAWKADSSPVKAGVETTTPSKQSNNKYAASSYLSLTPEQWKSHRSYSCQVTHEGSTVEKTVAPTEVS

SEQ ID NO: 27 - protein, 451 aa, Artificial Sequence
  Description of Artificial Sequence: Synthetic       polypeptide
EVQLLESGGGLVQPGGSLRLSCAASGFTFSSYAMSWVRQAPGKGLEWVSAISGSGGSTYYADSVKGRFTISRDNSKNTLYLQMNSLRAEDTAVYYCARGSYGTYYGNYFEYWGRGTLVTVSSASTKGPSVCPLAPSSKSTSGGTAALGCLVKDYFPEPVTVSWNSGALTSGVHTFPAVLQSSGLYSLSSVVTVPSSSLGTQTYICNVNHKPSNTKVDKRVEPKSVDKTHTCPPCPAPELLGGPSVFLFPPKPKDTLMISRTPEVTCVVVDVSHEDPEVKFNWYVDGVEVHNAKTKPREEQYNSTYRVVSVLTVLHQDWLNGKEYKCKVSNKALPAPIEKTISKAKGQPREPQVYTLPPCREEMTKNQVSLWCLVKGFYPSDIAVEWESNGQPENNYKTTPPVLDSDGSFFLYSKLTVDKSRWQQGNVFSCSVMHEALHNHYTQKSLSLSPG

SEQ ID NO: 28 - protein, 214 aa, Artificial Sequence
  Description of Artificial Sequence: Synthetic       polypeptide
SYVLTQPPSVSVAPGKTARITCGGDNIGGKSVHWYQQKPGQAPVLVIYYDSDRPSGIPERFSGSNSGNTATLTISRVEAGDEADYYCQVLDRRSDHFLFGGGTKLTVLGQPKAAPSVTLFPPCSEELQANKATLVCLISDFYPGAVTVAWKADSSPVKAGVETTTPSKQSNNKYAASSYLSLTPEQWKSHRSYSCQVTHEGSTVEKTVAPTEVS

SEQ ID NO: 29 - DNA, 642 bp, Artificial Sequence
  Description of Artificial Sequence: Synthetic polynucleotide
agctacgtgctgacgcagccgccgtcagtgtcagtggccccaggaaagacggccaggattacctgtgggggagacaacattggaggtaaaagtgttcactggtaccagcagaagccaggccaggcccctgtgttggtcatctattatgatagtgaccggccctcaggcatccctgagcgattctctggctccaactctgggaacacggccaccctgaccatcagcagggtcgaagccggggatgaggccgattattactgtcaggtgttggatcgtcgtagtgatcatttcctgttcggcggagggaccaagctgaccgtcctaggtcagcccaaggcggcgccctcggtcactctgttcccgccctgctctgaggagcttcaagccaacaaggccacactggtgtgtctcataagtgacttctacccgggagccgtgacagtggcctggaaggcagatagcagccccgtcaaggcgggagtggagaccaccacaccctccaaacaaagcaacaacaagtacgcggccagcagctacctgagcctgacgcctgagcagtggaagtcccacagaagctacagctgccaggtcacgcatgaagggagcaccgtggagaagacagtggcccctacagaagtgtca

SEQ ID NO: 30 - protein, 452 aa, Artificial Sequence
  Description of Artificial Sequence: Synthetic       polypeptide
EVQLLESGGGLVQPGGSLRLSCAASGFTFSSYAMSWVRQAPGKGLEWVSAISGSGGSTYYADSVKGRFTISRDNSKNTLYLQMNSLRAEDTAVYYCARGSYGTYYGNYFEYWGQGTLVTVSSASTKGPSVCPLAPSSKSTSGGTAALGCLVKDYFPEPVTVSWNSGALTSGVHTFPAVLQSSGLYSLSSVVTVPSSSLGTQTYICNVNHKPSNTKVDKRVEPKSVDKTHTCPPCPAPEFEGGPSVFLFPPKPKDTLMISRTPEVTCVVVDVSHEDPEVKFNWYVDGVEVHNAKTKPREEQYNSTYRVVSVLTVLHQDWLNGKEYKCKVSNKALPASIEKTISKAKGQPREPQVYTLPPCREEMTKNQVSLWCLVKGFYPSDIAVEWESNGQPENNYKTTPPVLDSDGSFFLYSKLTVDKSRWQQGNVFSCSVMHEALHNHYTQKSLSLSPGK

SEQ ID NO: 31 - DNA, 1356 bp, Artificial Sequence
  Description of Artificial Sequence: Synthetic polynucleotide
gaggtgcagctgttggagtctgggggaggcttggtacagcctggggggtccctgagactctcctgtgcagcctctggattcacctttagcagctatgccatgagctgggtccgccaggctccagggaaggggctggagtgggtctcagctattagtggtagtggtggtagcacatactacgcagactccgtgaagggccggttcaccatctccagagacaattccaagaacacgctgtatctgcaaatgaacagcctgagagccgaggacacggccgtgtattactgtgcgagagggtcctatggtacctactacggaaactactttgaatactggggccagggcaccctggtcaccgtctcgagtgcgtcgaccaaaggtccgagcgtgtgcccgctggcaccgagcagcaaaagcacctctggtggcaccgcagcactgggttgtctggtgaaagattattttccggaaccggttaccgtttcttggaatagcggtgcactgaccagcggtgttcatacctttccggcagtcctgcagagcagcggtctgtatagcctgtctagcgttgttaccgttccgagcagcagcctgggcacccagacctatatttgcaatgtgaatcataaaccgagcaataccaaagttgataaacgcgttgaaccgaaaagcgtggacaaaactcacacgtgcccaccgtgcccagcacctgagttcgaggggggaccgtcagtcttcctcttccccccaaaacccaaggacaccctcatgatctcccggacccctgaggtcacatgcgtggtggtggacgtgagccacgaagaccctgaggtcaagttcaactggtacgtggacggcgtggaggtgcataatgccaagacaaagccgcgggaggagcagtacaacagcacgtaccgtgtggtcagcgtcctcaccgtcctgcaccaggactggctgaatggcaaggagtacaagtgcaaggtctccaacaaagccctcccagccagcatcgagaaaaccatctccaaagccaaagggcagccccgagaaccacaggtctacaccctgcccccatgccgggaggagatgaccaagaaccaggtcagcctgtggtgcctggtcaaaggcttctatcccagcgacatcgccgtggagtgggagagcaatgggcagccggagaacaactacaagaccacgcctcccgtgctggactccgacggctccttcttcctctatagcaagctcaccgtggacaagagcaggtggcagcaggggaacgtcttctcatgctccgtgatgcatgaggctctgcacaaccactacacgcagaagagcttaagcctgtctccgggtaaa

SEQ ID NO: 32 - protein, 214 aa, Artificial Sequence
  Description of Artificial Sequence: Synthetic       polypeptide
DIQMTQSPSSLSASVGDRVTITCRASQDISNYLNWYQQKPGKAPKLLIYYTSKLHSGVPSRFSGSGSGTDYTLTISSLQPEDFATYYCQQGSALPWTFGQGTKVEIKRTVAAPSVFIFPPSDEQLKSGTASVVCLLNNFYPREAKVQWKVDNALQSGNSQESVTEQDSKDSTYSLSSTLTLSKADYEKHKVYACEVTHQGLSSPVTKSFNRGEC

SEQ ID NO: 33 - protein, 215 aa, Artificial Sequence; identical to SEQ ID NO: 15
  Description of Artificial Sequence: Synthetic       polypeptide

SEQ ID NO: 34 - protein, 707 aa, Artificial Sequence
  Description of Artificial Sequence: Synthetic       polypeptide
EIVLTQSPGTLSLSPGERATLSCRASQRVSSSYLAWYQQKPGQAPRLLIYDASSRATGIPDRFSGSGSGTDFTLTISRLEPEDFAVYYCQQYGSLPWTFGCGTKVEIKGGGGSGGGGSGGGGSGGGGSEVQLVESGGGLVQPGGSLRLSCAASGFTFSRYWMSWVRQAPGKCLEWVANIKQDGSEKYYVDSVKGRFTISRDNAKNSLYLQMNSLRAEDTAVYYCAREGGWFGELAFDYWGQGTLVTVSSGGGGSGGGGSQVQLQESGPGLVKPSQTLSLTCAVYGGSFSSGYWNWIRKHPGKGLEYIGYISYNGITYHNPSLKSRITINRDTSKNQYSLQLNSVTPEDTAVYYCARYKYDYDGGHAMDYWGQGTLVTVSSASTKGPSVFPLAPCSRSTSESTAALGCLVKDYFPEPVTVSWNSGALTSGVHTFPAVLQSSGLYSLSSVVTVPSSSLGTKTYTCNVDHKPSNTKVDKRVESKYGPPCPPCPAPEFLGGPSVFLFPPKPKDTLMISRTPEVTCVVVDVSQEDPEVQFNWYVDGVEVHNAKTKPREEQFNSTYRVVSVLTVLHQDWLNGKEYKCKVSNKGLPSSIEKTISKAKGQPREPQVYTLPPSQEEMTKNQVSLTCLVKGFYPSDIAVEWESNGQPENNYKTTPPVLDSDGSFFLYSRLTVDKSRWQEGNVFSCSVMHEALHNHYTQKSLSLSLGK

SEQ ID NO: 35 - protein, 707 aa, Artificial Sequence
  Description of Artificial Sequence: Synthetic       polypeptide
QVQLQESGPGLVKPSQTLSLTCAVYGGSFSSGYWNWIRKHPGKGLEYIGYISYNGITYHNPSLKSRITINRDTSKNQYSLQLNSVTPEDTAVYYCARYKYDYDGGHAMDYWGQGTLVTVSSASTKGPSVFPLAPCSRSTSESTAALGCLVKDYFPEPVTVSWNSGALTSGVHTFPAVLQSSGLYSLSSVVTVPSSSLGTKTYTCNVDHKPSNTKVDKRVESKYGPPCPPCPAPEFLGGPSVFLFPPKPKDTLMISRTPEVTCVVVDVSQEDPEVQFNWYVDGVEVHNAKTKPREEQFNSTYRVVSVLTVLHQDWLNGKEYKCKVSNKGLPSSIEKTISKAKGQPREPQVYTLPPSQEEMTKNQVSLTCLVKGFYPSDIAVEWESNGQPENNYKTTPPVLDSDGSFFLYSRLTVDKSRWQEGNVFSCSVMHEALHNHYTQKSLSLSLGKGGGGSGGGGSEIVLTQSPGTLSLSPGERATLSCRASQRVSSSYLAWYQQKPGQAPRLLIYDASSRATGIPDRFSGSGSGTDFTLTISRLEPEDFAVYYCQQYGSLPWTFGCGTKVEIKGGGGSGGGGSGGGGSGGGGSEVQLVESGGGLVQPGGSLRLSCAASGFTFSRYWMSWVRQAPGKCLEWVANIKQDGSEKYYVDSVKGRFTISRDNAKNSLYLQMNSLRAEDTAVYYCAREGGWFGELAFDYWGQGTLVTVSS

SEQ ID NO: 36 - protein, 707 aa, Artificial Sequence; identical to SEQ ID NO: 35
  Description of Artificial Sequence: Synthetic       polypeptide

SEQ ID NO: 37 - protein, 718 aa, Artificial Sequence
  Description of Artificial Sequence: Synthetic       polypeptide
EVQLVESGGGLVQPGGSLRLSCAASGFTFSSHDMHWVRQATGKGLEWVSGIGTAGDTYYPDSVKGRFTISRENAKNSLYLQMNSLRAGDTAVYYCARDRYSPTGHYYGMDVWGQGTTVTVSSASTKGPSVFPLAPSSKSTSGGTAALGCLVKDYFPEPVTVSWNSGALTSGVHTFPAVLQSSGLYSLSSVVTVPSSSLGTQTYICNVNHKPSNTKVDKRVEPKSCDKTHTCPPCPAPELLGGPSVFLFPPKPKDTLMISRTPEVTCVVVDVSHEDPEVKFNWYVDGVEVHNAKTKPREEQYNSTYRVVSVLTVLHQDWLNGKEYKCKVSNKALPAPIEKTISKAKGQPREPQVYTLPPSREEMTKNQVSLTCLVKGFYPSDIAVEWESNGGGGSGGGGSEIVMTQSPATLSVSPGERATLSCRASQSVSSYLGWYQQKPGQAPRLLIYGASTRATGIPARFSGSGSGTEFTLTISSLQSEDFAVYYCQQYQNWPLLTFGCGTKLEIKGGGGSGGGGSGGGGSGGGGSEVQLLESGGGLVQPGGSLRLSCAASGFTFSPYMMQWVRQAPGKCLEWVSSIWPSGGKTYYADSVKGRFTISRDNSKNTLYLQMNSLRAEDTAVYYCARVRRGGATDYWGQGTLVTVSSGGGGSGGGGSGQPENNYKTTPPVLDSDGSFFLYSKLTVDKSRWQQGNVFSCSVMHEALHNHYTQKSLSLSPGK

SEQ ID NO: 38 - protein, 716 aa, Artificial Sequence
  Description of Artificial Sequence: Synthetic       polypeptide
EVQLLESGGGLVQPGGSLRLSCAASGFTFSPYMMQWVRQAPGKGLEWVSSIWPSGGKTYYADSVKGRFTISRDNSKNTLYLQMNSLRAEDTAVYYCARVRRGGATDYWGQGTLVTVSSASTKGPSVFPLAPSSKSTSGGTAALGCLVKDYFPEPVTVSWNSGALTSGVHTFPAVLQSSGLYSLSSVVTVPSSSLGTQTYICNVNHKPSNTKVDKRVEPKSCDKTHTCPPCPAPELLGGPSVFLFPPKPKDTLMISRTPEVTCVVVDVSHEDPEVKFNWYVDGVEVHNAKTKPREEQYNSTYRVVSVLTVLHQDWLNGKEYKCKVSNKALPAPIEKTISKAKGQPREPQVYTLPPSREEMTKNQVSLTCLVKGFYPSDIAVEWESNGGGGSGGGGSDIQMTQSPSTLSASVGDRVTITCRASQSISSWLAWYQQKPGKAPKLLIYKASSLESGVPSRFSGSGSGTEFTLTISSLQPDDFATYYCKQYADYWTFGCGTKVEIKGGGGSGGGGSGGGGSGGGGSEVQLVESGGGLVQPGGSLRLSCAASGFTFSSHDMHWVRQATGKCLEWVSGIGTAGDTYYPDSVKGRFTISRENAKNSLYLQMNSLRAGDTAVYYCARDRYSPTGHYYGMDVWGQGTTVTVSSGGGGSGGGGSGQPENNYKTTPPVLDSDGSFFLYSKLTVDKSRWQQGNVFSCSVMHEALHNHYTQKSLSLSPGK

SEQ ID NO: 39 - protein, 5 aa, Artificial Sequence
  Description of Artificial Sequence: Synthetic       polypeptide
ISRTP

SEQ ID NO: 40 - protein, 5 aa, Artificial Sequence
  Description of Artificial Sequence: Synthetic       polypeptide
AKGQP

SEQ ID NO: 41 - protein, 10 aa, Artificial Sequence
  Description of Artificial Sequence: Synthetic       polypeptide
GGGGSGGGGS

SEQ ID NO: 42 - protein, 15 aa, Artificial Sequence
  Description of Artificial Sequence: Synthetic       polypeptide
GGGGSGGGGSGGGGS

SEQ ID NO: 43 - protein, 20 aa, Artificial Sequence
  Description of Artificial Sequence: Synthetic       polypeptide
GGGGSGGGGSGGGGSGGGGS

SEQ ID NO: 44 - protein, 15 aa, Artificial Sequence
  Description of Artificial Sequence: Synthetic       polypeptide
EPKSCDKTHTCPPCP

SEQ ID NO: 45 - protein, 8 aa, Artificial Sequence
  Description of Artificial Sequence: Synthetic       polypeptide
EPKSCDKT

SEQ ID NO: 46 - protein, 8 aa, Artificial Sequence
  Description of Artificial Sequence: Synthetic       polypeptide
EPKSCGKT

SEQ ID NO: 47 - protein, 5 aa, Artificial Sequence
  Description of Artificial Sequence: Synthetic       polypeptide
EPKSC

SEQ ID NO: 48 - protein, 5 aa, Artificial Sequence
  Description of Artificial Sequence: Synthetic       polypeptide
GGGGS

SEQ ID NO: 49 - protein, 112 aa, Artificial Sequence
  Description of Artificial Sequence: Synthetic       polypeptide
QIVLTQSPATLSLSPGERATLSCSASSKHTNLYWSRHMYWYQQKPGQAPRLLIYLTSNRATGIPARFSGSGSGTDFTLTISSLEPEDFAVYYCQQWSSNPFTFGQGTKLEIK

SEQ ID NO: 50 - protein, 449 aa, Artificial Sequence
  Description of Artificial Sequence: Synthetic       polypeptide
EVQLVESGGGLVQPGGSLRLSCAASGFTFSDYGMHWVRQAPGKGLEWVAYISSGSYTIYSADSVKGRFTISRDNAKNSLYLQMNSLRAEDTAVYYCARRAPNSFYEYYFDYWGQGTTVTVSSASTKGPSVFPLAPCSRSTSESTAALGCLVKDYFPEPVTVSWNSGALTSGVHTFPAVLQSSGLYSLSSVVTVPSSSLGTKTYTCNVDHKPSNTKVDKRVESKYGPPCPPCPAPEFLGGPSVFLFPPKPKDTLMISRTPEVTCVVVDVSQEDPEVQFNWYVDGVEVHNAKTKPREEQFNSTYRVVSVLTVLHQDWLNGKEYKCKVSNKGLPSSIEKTISKAKGQPREPQVYTLPPSQEEMTKNQVSLTCLVKGFYPSDIAVEWESNGQPENNYKTTPPVLDSDGSFFLYSRLTVDKSRWQEGNVFSCSVMHEALHNHYTQKSLSLSLGK

SEQ ID NO: 51 - protein, 122 aa, Artificial Sequence
  Description of Artificial Sequence: Synthetic       polypeptide
EVQLVESGGGLVQPGGSLRLSCAASGFTFSDYGMHWVRQAPGKGLEWVAYISSGSYTIYSADSVKGRFTISRDNAKNSLYLQMNSLRAEDTAVYYCARRAPNSFYEYYFDYWGQGTTVTVSS

SEQ ID NO: 52 - protein, 125 aa, Artificial Sequence
  Description of Artificial Sequence: Synthetic       polypeptide
QVQLVESGGGVVQPGRSLRLSCAASGFTFSSYGMHWVRQAPGKGLEWVAVIWYDGSNKYYADSVKGRFTISRDNSKNTLYLQMNSLRAEDTAVYYCARDPRGATLYYYYYGMDVWGQGTTVTVSS

SEQ ID NO: 53 - protein, 167 aa, Artificial Sequence
  CTLA-4 HC
GVVQPGRSLRLSCAASGFTFSSYGMHWVRQAPGKGLEWVAVIWYDGSNKYYADSVKGRFTISRDNSKNTLYLQMNSLRAEDTAVYYCARDPRGATLYYYYYGMDVWGQGTTVTVSSASTKGPSVFPLAPCSRSTSESTAALGCLVKDYFPEPVTVSWNSGALTSGVH

SEQ ID NO: 54 - protein, 107 aa, Artificial Sequence
  Description of Artificial Sequence: Synthetic       polypeptide
DIQMTQSPSSLSASVGDRVTITCRASQSINSYLDWYQQKPGKAPKLLIYAASSLQSGVPSRFSGSGSGTDFTLTISSLQPEDFATYYCQQYYSTPFTFGPGTKVEIK

SEQ ID NO: 55 - protein, 214 aa, Artificial Sequence
  Description of Artificial Sequence: Synthetic       polypeptide
DIQMTQSPSSLSASVGDRVTITCRASQSINSYLDWYQQKPGKAPKLLIYAASSLQSGVPSRFSGSGSGTDFTLTISSLQPEDFATYYCQQYYSTPFTFGPGTKVEIKRTVAAPSVFIFPPSDEQLKSGTASVVCLLNNFYPREAKVQWKVDNALQSGNSQESVTEQDSKDSTYSLSSTLTLSKADYEKHKVYACEVTHQGLSSPVTKSFNRGEC

SEQ ID NO: 56 - protein, 114 aa, Artificial Sequence
  Description of Artificial Sequence: Synthetic       polypeptide
EVQLVESGGGLVQPGRSLRLSCTASGYTFPDYYMNWVRQAPGKGLEWVGDIDPNYGGTTYNASVKGRFTISVDRSKSIAYLQMSSLKTEDTAVYYCARGALTDWGQGTMVTVSS

SEQ ID NO: 57 - protein, 213 aa, Artificial Sequence
  Description of Artificial Sequence: Synthetic       polypeptide
QIQLTQSPSILSASVGDRVTITCRASSSVSYIYWFQQKPGKAPKPLIYATFNLASGVPSRFSGSGSGTSYTLTISSLQPEDFATYYCQQWSNNPLTFGQGTKVEIKRTVAAPSVFIFPPSDEQLKSGTASVVCLLNNFYPREAKVQWKVDNALQSGNSQESVTEQDSKDSTYSLSSTLTLSKADYEKHKVYACEVTHQGLSSPVTKSFNRGEC

SEQ ID NO: 58 - protein, 106 aa, Artificial Sequence
  Description of Artificial Sequence: Synthetic       polypeptide
QIQLTQSPSILSASVGDRVTITCRASSSVSYIYWFQQKPGKAPKPLIYATFNLASGVPSRFSGSGSGTSYTLTISSLQPEDFATYYCQQWSNNPLTFGQGTKVEIK

SEQ ID NO: 59 - protein, 121 aa, Artificial Sequence
  Description of Artificial Sequence: Synthetic       polypeptide
EVQLVESGGGLVQPGGSLRLSCAASGFTFSRYWMSWVRQAPGKGLEWVANIKQDGSEKYYVDSVKGRFTISRDNAKNSLYLQMNSLRAEDTAVYYCAREGGWFGELAFDYWGQGTLVTVSS

SEQ ID NO: 60 - protein, 108 aa, Artificial Sequence
  Description of Artificial Sequence: Synthetic       polypeptide
EIVLTQSPGTLSLSPGERATLSCRASQRVSSSYLAWYQQKPGQAPRLLIYDASSRATGIPDRFSGSGSGTDFTLTISRLEPEDFAVYYCQQYGSLPWTFGQGTKVEIK

SEQ ID NO: 61 - protein, 214 aa, Artificial Sequence
  Description of Artificial Sequence: Synthetic       polypeptide
QTVLTQPPSVSVAPGKTASISCGGDNIGGKSVHWYQQKPGQAPVLVIYYDSDRPSGIPQRFSGSNSGNTATLTIHRVEAGDEADYYCQVLDRRSDHWLFGGGTKLTVLGQPKAAPSVTLFPPSSEELQANKATLVCLISDFYPGAVTVAWKADSSPVKAGVETTTPSKQSNNKYAASSYLSLTPEQWKSHRSYSCQVTHEGSTVEKTVAPTECS

SEQ ID NO: 62 - protein, 108 aa, Artificial Sequence
  Description of Artificial Sequence: Synthetic       polypeptide
QTVLTQPPSVSVAPGKTASISCGGDNIGGKSVHWYQQKPGQAPVLVIYYDSDRPSGIPQRFSGSNSGNTATLTIHRVEAGDEADYYCQVLDRRSDHWLFGGGTKLTVL

SEQ ID NO: 63 - protein, 449 aa, Artificial Sequence
  Description of Artificial Sequence: Synthetic       polypeptide
EVQLLESGGGLVQPGGSLRLSCAASGFTFSSYAMSWVRQAPGKGLEWVSAISGSGGSTYYADSVKGRFTISRDNSKNTLYLQMNSLRAEDTAVYYCARGSYGTYYGNYFEYWGRGTLVTVSSASTKGPSVFPLAPCSRSTSESTAALGCLVKDYFPEPVTVSWNSGALTSGVHTFPAVLQSSGLYSLSSVVTVPSSSLGTKTYTCNVDHKPSNTKVDKRVESKYGPPCPPCPAPEFLGGPSVFLFPPKPKDTLMISRTPEVTCVVVDVSQEDPEVQFNWYVDGVEVHNAKTKPREEQFNSTYRVVSVLTVLHQDWLNGKEYKCKVSNKGLPSSIEKTISKAKGQPREPQVYTLPPSQEEMTKNQVSLTCLVKGFYPSDIAVEWESNGQPENNYKTTPPVLDSDGSFFLYSRLTVDKSRWQEGNVFSCSVMHEALHNHYTQKSLSLSLGK

SEQ ID NO: 64 - protein, 122 aa, Artificial Sequence
  Description of Artificial Sequence: Synthetic       polypeptide
EVQLLESGGGLVQPGGSLRLSCAASGFTFSSYAMSWVRQAPGKGLEWVSAISGSGGSTYYADSVKGRFTISRDNSKNTLYLQMNSLRAEDTAVYYCARGSYGTYYGNYFEYWGRGTLVTVSS

SEQ ID NO: 65 - protein, 214 aa, Artificial Sequence
  Description of Artificial Sequence: Synthetic       polypeptide
SYVLTQPPSVSVAPGKTARITCGGDNIGGKSVHWYQQKPGQAPVLVIYYDSDRPSGIPERFSGSNSGNTATLTISRVEAGDEADYYCQVLDRRSDHWLFGGGTKLTVLGQPKAAPSVTLFPPSSEELQANKATLVCLISDFYPGAVTVAWKADSSPVKAGVETTTPSKQSNNKYAASSYLSLTPEQWKSHRSYSCQVTHEGSTVEKTVAPTECS

SEQ ID NO: 66 - protein, 108 aa, Artificial Sequence
  Description of Artificial Sequence: Synthetic       polypeptide
SYVLTQPPSVSVAPGKTARITCGGDNIGGKSVHWYQQKPGQAPVLVIYYDSDRPSGIPERFSGSNSGNTATLTISRVEAGDEADYYCQVLDRRSDHWLFGGGTKLTVL

SEQ ID NO: 67 - protein, 449 aa, Artificial Sequence
  Description of Artificial Sequence: Synthetic       polypeptide
EVQLLESGGGLVQPGGSLRLSCAASGFTFSSYAMSWVRQAPGKGLEWVSAISGSGGSTYYADSVKGRFTISRDNSKNTLYLQMNSLRAEDTAVYYCARGSYGTYYGNYFEYWGQGTLVTVSSASTKGPSVFPLAPCSRSTSESTAALGCLVKDYFPEPVTVSWNSGALTSGVHTFPAVLQSSGLYSLSSVVTVPSSSLGTKTYTCNVDHKPSNTKVDKRVESKYGPPCPPCPAPEFLGGPSVFLFPPKPKDTLMISRTPEVTCVVVDVSQEDPEVQFNWYVDGVEVHNAKTKPREEQFNSTYRVVSVLTVLHQDWLNGKEYKCKVSNKGLPSSIEKTISKAKGQPREPQVYTLPPSQEEMTKNQVSLTCLVKGFYPSDIAVEWESNGQPENNYKTTPPVLDSDGSFFLYSRLTVDKSRWQEGNVFSCSVMHEALHNHYTQKSLSLSLGK

SEQ ID NO: 68 - protein, 122 aa, Artificial Sequence
  Description of Artificial Sequence: Synthetic       polypeptide
EVQLLESGGGLVQPGGSLRLSCAASGFTFSSYAMSWVRQAPGKGLEWVSAISGSGGSTYYADSVKGRFTISRDNSKNTLYLQMNSLRAEDTAVYYCARGSYGTYYGNYFEYWGQGTLVTVSS

SEQ ID NO: 69 - protein, 121 aa, Artificial Sequence
  Description of Artificial Sequence: Synthetic       polypeptide
QVQLQESGPGLVKPSQTLSLTCAVYGGSFSSGYWNWIRKHPGKGLEYIGYISYNGITYHNPSLKSRITINRDTSKNQYSLQLNSVTPEDTAVYYCARYKYDYDGGHAMDYWGQGTLVTVSS

SEQ ID NO: 70 - protein, 107 aa, Artificial Sequence
  Description of Artificial Sequence: Synthetic       polypeptide
DIQMTQSPSSLSASVGDRVTITCRASQDISNYLNWYQQKPGKAPKLLIYYTSKLHSGVPSRFSGSGSGTDYTLTISSLQPEDFATYYCQQGSALPWTFGQGTKVEIK

SEQ ID NO: 71 - protein, 451 aa, Artificial Sequence
  Description of Artificial Sequence: Synthetic       polypeptide
QVQLQESGPGLVKPSQTLSLTCAVYGGSFSSGYWNWIRKHPGKGLEYIGYISYNGITYHNPSLKSRITINRDTSKNQYSLQLNSVTPEDTAVYYCARYKYDYDGGHAMDYWGQGTLVTVSSASTKGPSVFPLAPSSKSTSGGTAALGCLVKDYFPEPVTVSWNSGALTSGVHTFPAVLQSSGLYSLSSVVTVPSSSLGTQTYICNVNHKPSNTKVDKRVEPKSCDKTHTCPPCPAPELLGGPSVFLFPPKPKDTLMISRTPEVTCVVVDVSHEDPEVKFNWYVDGVEVHNAKTKPREEQYNSTYRVVSVLTVLHQDWLNGKEYKCKVSNKALPAPIEKTISKAKGQPREPQVYTLPPSREEMTKNQVSLTCLVKGFYPSDIAVEWESNGQPENNYKTTPPVLDSDGSFFLYSKLTVDKSRWQQGNVFSCSVMHEALHNHYTQKSLSLSPGK

SEQ ID NO: 72 - protein, 214 aa, Artificial Sequence; identical to SEQ ID NO: 32
  Description of Artificial Sequence: Synthetic       polypeptide

SEQ ID NO: 73 - protein, 288 aa, Homo sapiens
MQIPQAPWPVVWAVLQLGWRPGWFLDSPDRPWNPPTFSPALLVVTEGDNATFTCSFSNTSESFVLNWYRMSPSNQTDKLAAFPEDRSQPGQDCRFRVTQLPNGRDFHMSVVRARRNDSGTYLCGAISLAPKAQIKESLRAELRVTERRAEVPTAHPSPSPRPAGQFQTLVVGVVGGLLGSLVLLVWVLAVICSRAARGTIGARRTGQPLKEDPSAVPVFSVDYGELDFQWREKTPEPPVPCVPEQTEYATIVFPSGMGTSSPARRGSADGPRSAQPLRPEDGHCSWPL

SEQ ID NO: 74 - protein, 176 aa, Homo sapiens
MRIFAVFIFMTYWHLLNAPYNKINQRILVVDPVTSEHELTCQAEGYPKAEVIWTSSDHQVLSGKTTTTNSKREEKLFNVTSTLRINTTTNEIFYCTFRRLDPEENHTAELVIPELPLAHPPNERTHLVILGAILLCLGVALTFIFRLRKGRMMDVKKCGIQDTNSKKQSDTHLEET

SEQ ID NO: 75 - protein, 223 aa, Homo sapiens
MACLGFQRHKAQLNLATRTWPCTLLFFLLFIPVFCKAMHVAQPAVVLASSRGIASFVCEYASPGKATEVRVTVLRQADSQVTEVCAATYMMGNELTFLDDSICTGTSSGNQVNLTIQGLRAMDTGLYICKVELMYPPPYYLGIGNGTQIYVIDPEPCPDSDFLLWILAAVSSGLFFYSFLLTAVSLSKMLKKRSPLTTGVYVKMPPTEPECEKQFQPYFIPIN

SEQ ID NO: 76 - protein, 301 aa, Homo sapiens
MFSHLPFDCVLLLLLLLLTRSSEVEYRAEVGQNAYLPCFYTPAAPGNLVPVCWGKGACPVFECGNVVLRTDERDVNYWTSRYWLNGDFRKGDVSLTIENVTLADSGIYCCRIQIPGIMNDEKFNLKLVIKPAKVTPAPTRQRDFTAAFPRMLTTRGHGPAETQTLGSLPDINLTQISTLANELRDSRLANDLRDSGATIRIGIYIGAGICAGLALALIFGALIFKWYSHSKEKIQNLSLISLANLPPSGLANAVAEGIRSEENIYTIEENVYEVEEPNEYYCYVSSRQQPSQPLGCRFAMP

SEQ ID NO: 77 - protein, 278 aa, Homo sapiens
MGSPGMVLGLLVQIWALQEASSLSVQQGPNLLQVRQGSQATLVCQVDQATAWERLRVKWTKDGAILCQPYITNGSLSLGVCGPQGRLSWQAPSHLTLQLDPVSLNHSGAYVCWAAVEIPELEEAEGNITRLFVDPDDPTQNRNRIASFPGFLFVLLGVGSMGVAAIVWGAWFWGRRSCQQRDSGNAFYSNVLYRPRGAPKKSEDCSGEGKDQRGQSIYSTSFPQPAPRQPHLASRPCPSPRPCPSPRPGHPVSMVRVSPRPSPTQQPRPKGFPKVGEE

SEQ ID NO: 78 - protein, 277 aa, Homo sapiens
MCVGARRLGRGPCAALLLLGLGLSTVTGLHCVGDTYPSNDRCCHECRPGNGMVSRCSRSQNTVCRPCGPGFYNDVVSSKPCKPCTWCNLRSGSERKQLCTATQDTVCRCRAGTQPLDSYKPGVDCAPCPPGHFSPGDNQACKPWTNCTLAGKHTLQPASNSSDAICEDRDPPATQPQETQGPPARPITVQPTEAWPRTSQGPSTRPVEVPGGRAVAAILGLGLVLGLLGPLAILLALYLLRRDQRLPPDAHKPPGGGSFRTPIQEEQADAHSTLAKI

SEQ ID NO: 79 - protein, 10 aa, Artificial Sequence
  Description of Artificial Sequence: Synthetic       polypeptide
GFTFSSYAMS

SEQ ID NO: 80 - protein, 17 aa, Artificial Sequence
  Description of Artificial Sequence: Synthetic       polypeptide
AISGSGGSTYYADSVKG

SEQ ID NO: 81 - protein, 13 aa, Artificial Sequence
  Description of Artificial Sequence: Synthetic       polypeptide
GSYGTYYGNYFEY

SEQ ID NO: 82 - protein, 11 aa, Artificial Sequence
  Description of Artificial Sequence: Synthetic       polypeptide
GGDNIGGKSVH

SEQ ID NO: 83 - protein, 7 aa, Artificial Sequence
  Description of Artificial Sequence: Synthetic       polypeptide
YDSDRPS

SEQ ID NO: 84 - protein, 9 aa, Artificial Sequence
  Description of Artificial Sequence: Synthetic       polypeptide
QVLDRRSDH

SEQ ID NO: 85 - protein, 122 aa, Artificial Sequence; identical to SEQ ID NO: 64
  Description of Artificial Sequence: Synthetic       polypeptide

SEQ ID NO: 86 - protein, 108 aa, Artificial Sequence; identical to SEQ ID NO: 62
  Description of Artificial Sequence: Synthetic       polypeptide

SEQ ID NO: 87 - protein, 449 aa, Artificial Sequence; identical to SEQ ID NO: 63
  Description of Artificial Sequence: Synthetic       polypeptide

SEQ ID NO: 88 - protein, 214 aa, Artificial Sequence; identical to SEQ ID NO: 61
  Description of Artificial Sequence: Synthetic       polypeptide

SEQ ID NO: 89 - protein, 712 aa, Artificial Sequence
  BiS3 PD-1(LO115)/TIM3(O13-1) HC
EVQLVESGGGLVQPGGSLRLSCAASGFTFSDYGMHWVRQAPGKGLEWVAYISSGSYTIYSADSVKGRFTISRDNAKNSLYLQMNSLRAEDTAVYYCARRAPNSFYEYYFDYWGQGTTVTVSSASTKGPSVFPLAPSSKSTSGGTAALGCLVKDYFPEPVTVSWNSGALTSGVHTFPAVLQSSGLYSLSSVVTVPSSSLGTQTYICNVNHKPSNTKVDKRVEPKSCDKTHTCPPCPAPEFEGGPSVFLFPPKPKDTLMISRTPEVTCVVVDVSHEDPEVKFNWYVDGVEVHNAKTKPREEQYNSTYRVVSVLTVLHQDWLNGKEYKCKVSNKALPASIEKTISKAKGQPREPQVYTLPPSREEMTKNQVSLTCLVKGFYPSDIAVEWESNGQPENNYKTTPPVLDSDGSFFLYSKLTVDKSRWQQGNVFSCSVMHEALHNHYTQKSLSLSPGKGGGGSGGGGSEVQLLESGGGLVQPGGSLRLSCAASGFTFSSYAMSWVRQAPGKCLEWVSAISGSGGSTYYADSVKGRFTISRDNSKNTLYLQMNSLRAEDTAVYYCARGSYGTYYGNYFEYWGQGTLVTVSSGGGGSGGGGSGGGGSGGGGSSYVLTQPPSVSVAPGKTARITCGGDNIGGKSVHWYQQKPGQAPVLVIYYDSDRPSGIPERFSGSNSGNTATLTISRVEAGDEADYYCQVLDRRSDHFLFGCGTKLTVL

SEQ ID NO: 90 - protein, 219 aa, Artificial Sequence; identical to SEQ ID NO: 2
  BiS3 PD-1(LO115)/TIM3(O13-1) LC

SEQ ID NO: 91 - protein, 722 aa, Artificial Sequence
  BiS5 PD-1(LO115)/TIM3(O13-1) HC
EVQLVESGGGLVQPGGSLRLSCAASGFTFSDYGMHWVRQAPGKGLEWVAYISSGSYTIYSADSVKGRFTISRDNAKNSLYLQMNSLRAEDTAVYYCARRAPNSFYEYYFDYWGQGTTVTVSSASTKGPSVFPLAPSSKSTSGGTAALGCLVKDYFPEPVTVSWNSGALTSGVHTFPAVLQSSGLYSLSSVVTVPSSSLGTQTYICNVNHKPSNTKVDKRVEPKSCDKTHTCPPCPAPEFEGGPSVFLFPPKPKDTLMISRTPEVTCVVVDVSHEDPEVKFNWYVDGVEVHNAKTKPREEQYNSTYRVVSVLTVLHQDWLNGKEYKCKVSNKALPASIEKTISKAKGQPREPQVYTLPPSREEMTKNQVSLTCLVKGFYPSDIAVEWESNGGGGSGGGGSEVQLLESGGGLVQPGGSLRLSCAASGFTFSSYAMSWVRQAPGKCLEWVSAISGSGGSTYYADSVKGRFTISRDNSKNTLYLQMNSLRAEDTAVYYCARGSYGTYYGNYFEYWGQGTLVTVSSGGGGSGGGGSGGGGSGGGGSSYVLTQPPSVSVAPGKTARITCGGDNIGGKSVHWYQQKPGQAPVLVIYYDSDRPSGIPERFSGSNSGNTATLTISRVEAGDEADYYCQVLDRRSDHFLFGCGTKLTVLGGGGSGGGGSGQPENNYKTTPPVLDSDGSFFLYSKLTVDKSRWQQGNVFSCSVMHEALHNHYTQKSLSLSPGK

SEQ ID NO: 92 - protein, 219 aa, Artificial Sequence; identical to SEQ ID NO: 2
  BiS5 PD-1(LO115)/TIM3(O13-1) LC

SEQ ID NO: 93 - protein, 214 aa, Artificial Sequence; identical to SEQ ID NO: 32
  OX40SLR LCv kappa

SEQ ID NO: 94 - protein, 720 aa, Artificial Sequence
  BiS5-OX40SLR HC-G1-N434A-PD-L1
QVQLQESGPGLVKPSQTLSLTCAVYGGSFSSGYWNWIRKHPGKGLEYIGYISYNAITYHNPSLKSRITINRDTSKNQYSLQLNSVTPEDTAVYYCARYKYDYEGGHAMDYWGQGTLVTVSSASTKGPSVFPLAPSSKSTSGGTAALGCLVKDYFPEPVTVSWNSGALTSGVHTFPAVLQSSGLYSLSSVVTVPSSSLGTQTYICNVNHKPSNTKVDKRVEPKSCDKTHTCPPCPAPELLGGPSVFLFPPKPKDTLMISRTPEVTCVVVDVSHEDPEVKFNWYVDGVEVHNAKTKPREEQYNSTYRVVSVLTVLHQDWLNGKEYKCKVSNKALPAPIEKTISKAKGQPREPQVYTLPPSREEMTKNQVSLTCLVKGFYPSDIAVEWESNGGGGSGGGGSEVQLVESGGGLVQPGGSLRLSCAASGFTFSRYWMSWVRQAPGKCLEWVANIKQDGSEKYYVDSVKGRFTISRDNAKNSLYLQMNSLRAEDTAVYYCAREGGWFGELAFDYWGQGTLVTVSSGGGGSGGGGSGGGGSGGGGSEIVLTQSPGTLSLSPGERATLSCRASQRVSSSYLAWYQQKPGQAPRLLIYDASSRATGIPDRFSGSGSGTDFTLTISRLEPEDFAVYYCQQYGSLPWTFGCGTKVEIKGGGGSGGGGSGQPENNYKTTPPVLDSDGSFFLYSKLTVDKSRWQQGNVFSCSVMHEALHAHYTQKSLSLSPGK

SEQ ID NO: 95 - protein, 707 aa, Artificial Sequence
  BiS2-PD-1- OX40 HC -4P
DIQMTQSPSSLSASVGDRVTITCRASQDISNYLNWYQQKPGKAPKLLIYYTSKLHSGVPSRFSGSGSGTDYTLTISSLQPEDFATYYCQQGSALPWTFGCGTKVEIKGGGGSGGGGSGGGGSGGGGSQVQLQESGPGLVKPSQTLSLTCAVYGGSFSSGYWNWIRKHPGKCLEYIGYISYNGITYHNPSLKSRITINRDTSKNQYSLQLNSVTPEDTAVYYCARYKYDYDGGHAMDYWGQGTLVTVSSGGGGSGGGGSEVQLVESGGGLVQPGGSLRLSCAASGFTFSDYGMHWVRQAPGKGLEWVAYISSGSYTIYSADSVKGRFTISRDNAKNSLYLQMNSLRAEDTAVYYCARRAPNSFYEYYFDYWGQGTTVTVSSASTKGPSVFPLAPCSRSTSESTAALGCLVKDYFPEPVTVSWNSGALTSGVHTFPAVLQSSGLYSLSSVVTVPSSSLGTKTYTCNVDHKPSNTKVDKRVESKYGPPCPPCPAPEFLGGPSVFLFPPKPKDTLMISRTPEVTCVVVDVSQEDPEVQFNWYVDGVEVHNAKTKPREEQFNSTYRVVSVLTVLHQDWLNGKEYKCKVSNKGLPSSIEKTISKAKGQPREPQVYTLPPSQEEMTKNQVSLTCLVKGFYPSDIAVEWESNGQPENNYKTTPPVLDSDGSFFLYSRLTVDKSRWQEGNVFSCSVMHEALHNHYTQKSLSLSLGK

SEQ ID NO: 96 - protein, 707 aa, Artificial Sequence
  BiS3-OX40 HC-4P-PD-1
EVQLVESGGGLVQPGGSLRLSCAASGFTFSDYGMHWVRQAPGKGLEWVAYISSGSYTIYSADSVKGRFTISRDNAKNSLYLQMNSLRAEDTAVYYCARRAPNSFYEYYFDYWGQGTTVTVSSASTKGPSVFPLAPCSRSTSESTAALGCLVKDYFPEPVTVSWNSGALTSGVHTFPAVLQSSGLYSLSSVVTVPSSSLGTKTYTCNVDHKPSNTKVDKRVESKYGPPCPPCPAPEFLGGPSVFLFPPKPKDTLMISRTPEVTCVVVDVSQEDPEVQFNWYVDGVEVHNAKTKPREEQFNSTYRVVSVLTVLHQDWLNGKEYKCKVSNKGLPSSIEKTISKAKGQPREPQVYTLPPSQEEMTKNQVSLTCLVKGFYPSDIAVEWESNGQPENNYKTTPPVLDSDGSFFLYSRLTVDKSRWQEGNVFSCSVMHEALHNHYTQKSLSLSLGKGGGGSGGGGSDIQMTQSPSSLSASVGDRVTITCRASQDISNYLNWYQQKPGKAPKLLIYYTSKLHSGVPSRFSGSGSGTDYTLTISSLQPEDFATYYCQQGSALPWTFGCGTKVEIKGGGGSGGGGSGGGGSGGGGSQVQLQESGPGLVKPSQTLSLTCAVYGGSFSSGYWNWIRKHPGKCLEYIGYISYNGITYHNPSLKSRITINRDTSKNQYSLQLNSVTPEDTAVYYCARYKYDYDGGHAMDYWGQGTLVTVSS

SEQ ID NO: 97 - protein, 219 aa, Artificial Sequence; identical to SEQ ID NO: 2
  PD1 LCv kappa